European Patent Specification EP 3 996 814 B1, published September 17, 2025. Title: Uso di un estratto di erbe comprendente verbascoside e aucubina per il trattamento di osteoartrite del ginocchio. Applicant: LABIOTRE S.R.L. The sequence listing filed with the application follows.

SEQUENCE LISTING (6 sequences)

SEQ ID NO: 1 - DNA, 21 bp, Artificial Sequence
  Primer for human COX-1
cgccagtgaatccctgttgtt

SEQ ID NO: 2 - DNA, 21 bp, Artificial Sequence
  Primer for human COX-1 (reverse)
aaggtggcattgacaaactcc

SEQ ID NO: 3 - DNA, 19 bp, Artificial Sequence
  Primer for human COX-2
ctggcgctcagccatacag

SEQ ID NO: 4 - DNA, 23 bp, Artificial Sequence
  Primer for human COX-2 (reverse)
cgcacttatactggtcaaatccc

SEQ ID NO: 5 - DNA, 21 bp, Artificial Sequence
  Primer for glyceraldehyde 3-phosphate dehydrogenase (GAPDH; gene housekeeping)
ggagcgagatccctccaaaat

SEQ ID NO: 6 - DNA, 23 bp, Artificial Sequence
  Primer for glyceraldehyde 3-phosphate dehydrogenase (GAPDH; gene housekeeping) (reverse)
ggctgttgtcatacttctcatgg